European Patent Application EP 4 238 991 A1, published September 6, 2023. Title: Anti-TIGIT Antibody or Antigen-Binding Fragment Thereof. Applicant: GUANGDONG FAPON BIOPHARMA INC. The sequence listing filed with the application follows.

SEQUENCE LISTING (98 sequences)

SEQ ID NO: 1 - protein, 5 aa, artificial sequence
  Synthesized
SYWMN

SEQ ID NO: 2 - protein, 17 aa, artificial sequence
  Synthesized
MIRPSDSETRLNQMFKD

SEQ ID NO: 3 - protein, 9 aa, artificial sequence
  Synthesized
IHDYGHGAY

SEQ ID NO: 4 - protein, 5 aa, artificial sequence
  Synthesized
DYFMD

SEQ ID NO: 5 - protein, 17 aa, artificial sequence
  Synthesized
RLNPNNGRTSYNQKFKG

SEQ ID NO: 6 - protein, 10 aa, artificial sequence
  Synthesized
GDLGRWYFDV

SEQ ID NO: 7 - protein, 5 aa, artificial sequence
  Synthesized
SYWIE

SEQ ID NO: 8 - protein, 17 aa, artificial sequence
  Synthesized
EILSGSGRTYFNEKFKG

SEQ ID NO: 9 - protein, 11 aa, artificial sequence
  Synthesized
RGLRGPYYFDY

SEQ ID NO: 10 - protein, 5 aa, artificial sequence
  Synthesized
DYNMH

SEQ ID NO: 11 - protein, 17 aa, artificial sequence
  Synthesized
YVNSFNGNTGYSQKFKS

SEQ ID NO: 12 - protein, 8 aa, artificial sequence
  Synthesized
SSRGGFAY

SEQ ID NO: 13 - protein, 6 aa, artificial sequence
  Synthesized
SDYAWN

SEQ ID NO: 14 - protein, 16 aa, artificial sequence
  Synthesized
YISYSGSTRSNPSLKS

SEQ ID NO: 15 - protein, 11 aa, artificial sequence
  Synthesized
WEVRNYYAMDY

SEQ ID NO: 16 - protein, 5 aa, artificial sequence
  Synthesized
DTYIH

SEQ ID NO: 17 - protein, 17 aa, artificial sequence
  Synthesized
GIGPANGNTKFDPKFQG

SEQ ID NO: 18 - protein, 10 aa, artificial sequence
  Synthesized
LLLRFYVLAY

SEQ ID NO: 19 - protein, 5 aa, artificial sequence
  Synthesized
NYWIG

SEQ ID NO: 20 - protein, 17 aa, artificial sequence
  Synthesized
DIYPGGGYTNYDEKFKG

SEQ ID NO: 21 - protein, 12 aa, artificial sequence
  Synthesized
GGYGSTYGYFDV

SEQ ID NO: 22 - protein, 11 aa, artificial sequence
  Synthesized
RASENIYSNLA

SEQ ID NO: 23 - protein, 7 aa, artificial sequence
  Synthesized
AASHLPD

SEQ ID NO: 24 - protein, 9 aa, artificial sequence
  Synthesized
QHFWGTPRT

SEQ ID NO: 25 - protein, 10 aa, artificial sequence
  Synthesized
SASSSVSYMH

SEQ ID NO: 26 - protein, 7 aa, artificial sequence
  Synthesized
DTSKLAS

SEQ ID NO: 27 - protein, 9 aa, artificial sequence
  Synthesized
QQWSSNSLT

SEQ ID NO: 28 - protein, 15 aa, artificial sequence
  Synthesized
RASKSVSTSGYSYMH

SEQ ID NO: 29 - protein, 7 aa, artificial sequence
  Synthesized
LVSNLES

SEQ ID NO: 30 - protein, 8 aa, artificial sequence
  Synthesized
QHIRELTR

SEQ ID NO: 31 - protein, 10 aa, artificial sequence
  Synthesized
SASSSVSYMH

SEQ ID NO: 32 - protein, 7 aa, artificial sequence
  Synthesized
DTSKLAS

SEQ ID NO: 33 - protein, 9 aa, artificial sequence
  Synthesized
QQWSSNSLT

SEQ ID NO: 34 - protein, 11 aa, artificial sequence
  Synthesized
KASQHVSTAVA

SEQ ID NO: 35 - protein, 7 aa, artificial sequence
  Synthesized
SASYRYT

SEQ ID NO: 36 - protein, 9 aa, artificial sequence
  Synthesized
QQHYNTPWT

SEQ ID NO: 37 - protein, 15 aa, artificial sequence
  Synthesized
RASKSVSTSGYSYMH

SEQ ID NO: 38 - protein, 7 aa, artificial sequence
  Synthesized
LVSNLES

SEQ ID NO: 39 - protein, 8 aa, artificial sequence
  Synthesized
QHIRELTR

SEQ ID NO: 40 - protein, 17 aa, artificial sequence
  Synthesized
KSSQSLLFSSDQKNYLA

SEQ ID NO: 41 - protein, 7 aa, artificial sequence
  Synthesized
WASTRES

SEQ ID NO: 42 - protein, 9 aa, artificial sequence
  Synthesized
QQYHKYPFT

SEQ ID NO: 43 - protein, 30 aa, artificial sequence
  Synthesized
QVQLQQPGAELVRPGASVKLSCKASGYSFT

SEQ ID NO: 44 - protein, 14 aa, artificial sequence
  Synthesized
WVKQRPGQGLEWIG

SEQ ID NO: 45 - protein, 32 aa, artificial sequence
  Synthesized
KATLTVDKSSSTAYMQLSSPTSDDSAVYYCAG

SEQ ID NO: 46 - protein, 11 aa, artificial sequence
  Synthesized
WGQGTLVTVSA

SEQ ID NO: 47 - protein, 30 aa, artificial sequence
  Synthesized
EVQLQQSGPELVKPGASVKMSCKASGFTFT

SEQ ID NO: 48 - protein, 14 aa, artificial sequence
  Synthesized
WVKQSRGASFEWIG

SEQ ID NO: 49 - protein, 32 aa, artificial sequence
  Synthesized
KATLTVDKSSSTAYMELNSLTSEDSAVYYCAR

SEQ ID NO: 50 - protein, 11 aa, artificial sequence
  Synthesized
WGAGTTVTVSS

SEQ ID NO: 51 - protein, 30 aa, artificial sequence
  Synthesized
QVQLQQSGAELMKPGASVKISCKATGYTFS

SEQ ID NO: 52 - protein, 14 aa, artificial sequence
  Synthesized
WVKQRPGHGLEWIG

SEQ ID NO: 53 - protein, 32 aa, artificial sequence
  Synthesized
KATFTADTSSNTSYMQLSSLTSEDSAVYFCAR

SEQ ID NO: 54 - protein, 11 aa, artificial sequence
  Synthesized
WGQGTTLTVSS

SEQ ID NO: 55 - protein, 30 aa, artificial sequence
  Synthesized
EVQLQQSGPELVKPGASVKISCKASGYTFT

SEQ ID NO: 56 - protein, 14 aa, artificial sequence
  Synthesized
WVKQSLGKSLEWIG

SEQ ID NO: 57 - protein, 32 aa, artificial sequence
  Synthesized
KVTLTVDRSSRTAYMDLRSLTSEDSAVFYCAR

SEQ ID NO: 58 - protein, 11 aa, artificial sequence
  Synthesized
WGQGTLVTVSA

SEQ ID NO: 59 - protein, 30 aa, artificial sequence
  Synthesized
DVQLQESGPGLVKPSQSLSLTCTVTGYSIT

SEQ ID NO: 60 - protein, 14 aa, artificial sequence
  Synthesized
WIRQFPGNKLEWMG

SEQ ID NO: 61 - protein, 32 aa, artificial sequence
  Synthesized
RISITRDTSKNQFFLQLNSMTAEDTATYYCGG

SEQ ID NO: 62 - protein, 11 aa, artificial sequence
  Synthesized
WGQGTSVTVSS

SEQ ID NO: 63 - protein, 30 aa, artificial sequence
  Synthesized
EVQLQQSGAELVKPGASVKLSCTASGFNIK

SEQ ID NO: 64 - protein, 14 aa, artificial sequence
  Synthesized
WVKQRPDQGLEWIG

SEQ ID NO: 65 - protein, 32 aa, artificial sequence
  Synthesized
KATITADTSSNTAYLQLSGLTSEDTAVYYCAK

SEQ ID NO: 66 - protein, 11 aa, artificial sequence
  Synthesized
WGQGTSVTVSS

SEQ ID NO: 67 - protein, 30 aa, artificial sequence
  Synthesized
QVQLQQSGAELVRPGTSVKMSCKAAGYTFT

SEQ ID NO: 68 - protein, 14 aa, artificial sequence
  Synthesized
WVKQRPGHGLEWIG

SEQ ID NO: 69 - protein, 32 aa, artificial sequence
  Synthesized
KATLTADTSSRTAYMQLSSLTSEDSAIYHCVN

SEQ ID NO: 70 - protein, 11 aa, artificial sequence
  Synthesized
WGAGTTVTVSS

SEQ ID NO: 71 - protein, 23 aa, artificial sequence
  Synthesized
DIQMIQSPASLSVSVGETVTITC

SEQ ID NO: 72 - protein, 15 aa, artificial sequence
  Synthesized
WYQQKQGKSPQLLVY

SEQ ID NO: 73 - protein, 32 aa, artificial sequence
  Synthesized
GVPSRFSGSGSGTQYSLKINSLQSEDFGSYYC

SEQ ID NO: 74 - protein, 11 aa, artificial sequence
  Synthesized
FGGGTKLEIKR

SEQ ID NO: 75 - protein, 23 aa, artificial sequence
  Synthesized
QIVLTQSPAIMSASPGEKVTMTC

SEQ ID NO: 76 - protein, 15 aa, artificial sequence
  Synthesized
WYQQKSGTSPKRWIY

SEQ ID NO: 77 - protein, 32 aa, artificial sequence
  Synthesized
GVPTRFSGSGSGTSYSLTISSMEAEDAASYFC

SEQ ID NO: 78 - protein, 11 aa, artificial sequence
  Synthesized
FGAGTKLELKR

SEQ ID NO: 79 - protein, 23 aa, artificial sequence
  Synthesized
DIVLTQSPASLAVSLGQRATISY

SEQ ID NO: 80 - protein, 15 aa, artificial sequence
  Synthesized
WNQQKPGQPPRLLIY

SEQ ID NO: 81 - protein, 32 aa, artificial sequence
  Synthesized
GVPARFSGSGSGTDFTLNIHPVEEEDAATYYC

SEQ ID NO: 82 - protein, 11 aa, artificial sequence
  Synthesized
SGGGTKLEIKR

SEQ ID NO: 83 - protein, 23 aa, artificial sequence
  Synthesized
QIVLTQSPAIMSASPGEKVTMTC

SEQ ID NO: 84 - protein, 15 aa, artificial sequence
  Synthesized
WYQQKSGTSPKRWIY

SEQ ID NO: 85 - protein, 32 aa, artificial sequence
  Synthesized
GVPARFSGSVSGTSYSLTISSMEAEDAATYYC

SEQ ID NO: 86 - protein, 11 aa, artificial sequence
  Synthesized
FGAGTKLELKR

SEQ ID NO: 87 - protein, 23 aa, artificial sequence
  Synthesized
DIVMTQSHKFMSTSVGDRVSITC

SEQ ID NO: 88 - protein, 15 aa, artificial sequence
  Synthesized
WYQQKPGQSPKLLIY

SEQ ID NO: 89 - protein, 32 aa, artificial sequence
  Synthesized
GVPDRFTGSGSGTDFTFTISSVQAEDLAVYYC

SEQ ID NO: 90 - protein, 11 aa, artificial sequence
  Synthesized
FGGGTKLEIKR

SEQ ID NO: 91 - protein, 23 aa, artificial sequence
  Synthesized
DIVLTQSPASLAVSLGQRATISY

SEQ ID NO: 92 - protein, 15 aa, artificial sequence
  Synthesized
WNQQKPGQPPRLLIY

SEQ ID NO: 93 - protein, 32 aa, artificial sequence; identical to SEQ ID NO: 81
  Synthesized

SEQ ID NO: 94 - protein, 11 aa, artificial sequence
  Synthesized
SGGGTKLEIKR

SEQ ID NO: 95 - protein, 23 aa, artificial sequence
  Synthesized
DIVMSQSPSSLPVSVGEKVTMSC

SEQ ID NO: 96 - protein, 15 aa, artificial sequence
  Synthesized
WYQQKPGQSPKLLIY

SEQ ID NO: 97 - protein, 32 aa, artificial sequence
  Synthesized
GVPDRLTGSGSGTDFTLTISSVKAEDLAVYYC

SEQ ID NO: 98 - protein, 11 aa, artificial sequence
  Synthesized
FGGGTKLEIKR